European Patent Specification EP 3 899 034 B1, published March 18, 2026. Title: Methods for RNA analysis. Applicant: CureVac AG. The sequence listing filed with the application follows.

SEQUENCE LISTING (11 sequences)

SEQ ID NO: 1 - RNA, 646 nt, Artificial Sequence
  R4032
gggagaaagcuuaccaugggcgcccccacccugccgccggccuggcagccguuccucaaggaccaccgcaucucgaccuucaagaacuggccguuccuggagggcugcgcgugcaccccggagcggauggccgaggccggcuucauccacugccccaccgagaacgagccggaccuggcccagugcuucuucugcuucaaggagcuggagggcugggagccggacgacgacccgaucgaggagcacaagaagcacagcagcggcugcgccuuccugagcgugaagaagcaguucgaggagcugacgcucggggaguuccugaagcuggaccgggagcgggccaagaacaagaucgcgaaggagaccaacaacaagaagaaggaguucgaggagaccgccaagaaggugcggcgggccaucgagcagcuggccgccauggacugaccacuaguuauaagacugacuagcccgaugggccucccaacgggcccuccuccccuccuugcaccgagauuaauaaaaaaaaaaaaaaaaaaaaaaaaaaaaaaaaaaaaaaaaaaaaaaaaaaaaaaaaaaaaaaaaugcaucccccccccccccccccccccccccccccccaaaggcucuuuucagagccaccagaauu

SEQ ID NO: 2 - DNA, 15 bp, Artificial Sequence
  5'-cutter
cggctcccagccctc

SEQ ID NO: 3 - DNA, 15 bp, Artificial Sequence
  5'-cutter
ggtaagctttctccc

SEQ ID NO: 4 - DNA, 19 bp, Artificial Sequence
  5'-cutter
ctcggtgcaaggaggggag

SEQ ID NO: 5 - RNA, 222 nt, Artificial Sequence
  R4032 expected 222 nt fragment
gggagaaagcuuaccaugggcgcccccacccugccgccggccuggcagccguuccucaaggaccaccgcaucucgaccuucaagaacuggccguuccuggagggcugcgcgugcaccccggagcggauggccgaggccggcuucauccacugccccaccgagaacgagccggaccuggcccagugcuucuucugcuucaaggagcuggagggcugggagccg

SEQ ID NO: 6 - RNA, 424 nt, Artificial Sequence
  R4032 expected 424 nt fragment
gacgacgacccgaucgaggagcacaagaagcacagcagcggcugcgccuuccugagcgugaagaagcaguucgaggagcugacgcucggggaguuccugaagcuggaccgggagcgggccaagaacaagaucgcgaaggagaccaacaacaagaagaaggaguucgaggagaccgccaagaaggugcggcgggccaucgagcagcuggccgccauggacugaccacuaguuauaagacugacuagcccgaugggccucccaacgggcccuccuccccuccuugcaccgagauuaauaaaaaaaaaaaaaaaaaaaaaaaaaaaaaaaaaaaaaaaaaaaaaaaaaaaaaaaaaaaaaaaaugcaucccccccccccccccccccccccccccccccaaaggcucuuuucagagccaccagaauu

SEQ ID NO: 7 - RNA, 512 nt, Artificial Sequence
  R4032 expected 512 nt fragment
gggagaaagcuuaccaugggcgcccccacccugccgccggccuggcagccguuccucaaggaccaccgcaucucgaccuucaagaacuggccguuccuggagggcugcgcgugcaccccggagcggauggccgaggccggcuucauccacugccccaccgagaacgagccggaccuggcccagugcuucuucugcuucaaggagcuggagggcugggagccggacgacgacccgaucgaggagcacaagaagcacagcagcggcugcgccuuccugagcgugaagaagcaguucgaggagcugacgcucggggaguuccugaagcuggaccgggagcgggccaagaacaagaucgcgaaggagaccaacaacaagaagaaggaguucgaggagaccgccaagaaggugcggcgggccaucgagcagcuggccgccauggacugaccacuaguuauaagacugacuagcccgaugggccucccaacgggcccuccuccccuccuugcaccgag

SEQ ID NO: 8 - RNA, 134 nt, Artificial Sequence
  R4032 expected 134 nt fragment
auuaauaaaaaaaaaaaaaaaaaaaaaaaaaaaaaaaaaaaaaaaaaaaaaaaaaaaaaaaaaaaaaaaaugcaucccccccccccccccccccccccccccccccaaaggcucuuuucagagccaccagaauu

SEQ ID NO: 9 - RNA, 15 nt, Artificial Sequence
  Example  target sequence
gggagaaagcuuacc

SEQ ID NO: 10 - DNA, 15 bp, Artificial Sequence
  Example complement target sequence
ggtaagcttactccc

SEQ ID NO: 11 - RNA, 15 nt, Artificial Sequence
  Example target sequence (w is a or u)
  misc_feature (7)..(7): w is a or u
gggagawagcuuacc